European Patent Application EP 4 707 300 A1, published March 11, 2026. Title: ANTI-HUMAN IL-15 ANTIBODY AND USE THEREOF. Applicant: Beijing Wisdomab Biotechnology Co., Ltd. The sequence listing filed with the application follows.

SEQUENCE LISTING (51 sequences)

SEQ ID NO: 1 - protein, 114 aa, Homo sapiens
NWVNVISDLKKIEDLIQSMHIDATLYTESDVHPSCKVTAMKCFLLELQVISLESGDASIHDTVENLIILANNSLSSNGNVTESGCKECEELEEKNIKEFLQSFVHIVQMFINTS

SEQ ID NO: 2 - protein, 98 aa, Homo sapiens
ITCPPPMSVEHADIWVKSYSLYSRERYICNSGFKRKAGTSSLTECVLNKATNVAHWTTPSLKCIRDPALVHQRPAPPSTVTTAGVTPQPESLSPSGKE

SEQ ID NO: 3 - protein, 114 aa, Macaca fascicularis
NWVNVISDLKKIEDLIQSMHIDATLYTESDVHPSCKVTAMKCFLLELQVISHESGDTDIHDTVENLIILANNILSSNGNITESGCKECEELEEKNIKEFLQSFVHIVQMFINTS

SEQ ID NO: 4 - protein, 98 aa, Macaca fascicularis
ITCPPPVSVEHADIRVKSYSLYSRERYICNSGFKRKAGTSSLTECVLNKATNIAHWTTPSLKCIRDPLLARQRPAPPFTVTTAGVTPQPESLSPSGKE

SEQ ID NO: 5 - protein, 114 aa, Mus musculus
NWIDVRYDLEKIESLIQSIHIDTTLYTDSDFHPSCKVTAMNCFLLELQVILHEYSNMTLNETVRNVLYLANSTLSSNKNVAESGCKECEELEEKTFTEFLQSFIRIVQMFINTS

SEQ ID NO: 6 - protein, 97 aa, Mus musculus
GTTCPPPVSIEHADIRVKNYSVNSRERYVCNSGFKRKAGTSTLIECVINKNTNVAHWTTPSLKCIRDPSLAHYSPVPTVVTPKVTSQPESPSPSAKE

SEQ ID NO: 7 - protein, 6 aa, synthetic construct
HHHHHH

SEQ ID NO: 8 - protein, 229 aa, synthetic construct
ASVPRDSGCKPCICTVPEVSSVFIFPPKPKDVLTITLTPKVTCVVVDISKDDPEVQFSWFVDDVEVHTAQTQPREEQFNSTFRSVSELPIMHQDWLNGKEFKCRVNSAAFPAPIEKTISKTKGRPKAPQVYTIPPPKEQMAKDKVSLTCMITDFFPEDITVEWQWNGQPAENYKNTQPIMDTDGSYFVYSKLNVQKSNWEAGNTFTCSVLHEGLHNHHTEKSLSHSPGK

SEQ ID NO: 9 - protein, 330 aa, Homo sapiens
ASTKGPSVFPLAPSSKSTSGGTAALGCLVKDYFPEPVTVSWNSGALTSGVHTFPAVLQSSGLYSLSSVVTVPSSSLGTQTYICNVNHKPSNTKVDKRVEPKSCDKTHTCPPCPAPELLGGPSVFLFPPKPKDTLMISRTPEVTCVVVDVSHEDPEVKFNWYVDGVEVHNAKTKPREEQYNSTYRVVSVLTVLHQDWLNGKEYKCKVSNKALPAPIEKTISKAKGQPREPQVYTLPPSREEMTKNQVSLTCLVKGFYPSDIAVEWESNGQPENNYKTTPPVLDSDGSFFLYSKLTVDKSRWQQGNVFSCSVMHEALHNHYTQKSLSLSPGK

SEQ ID NO: 10 - protein, 330 aa, synthetic construct
ASTKGPSVFPLAPSSKSTSGGTAALGCLVKDYFPEPVTVSWNSGALTSGVHTFPAVLQSSGLYSLSSVVTVPSSSLGTQTYICNVNHKPSNTKVDKRVEPKSCDKTHTCPPCPAPEFEGGPSVFLFPPKPKDTLMISRTPEVTCVVVDVSHEDPEVKFNWYVDGVEVHNAKTKPREEQYNSTYRVVSVLTVLHQDWLNGKEYKCKVSNKALPASIEKTISKAKGQPREPQVYTLPPSREEMTKNQVSLTCLVKGFYPSDIAVEWESNGQPENNYKTTPPVLDSDGSFFLYSKLTVDKSRWQQGNVFSCSVMHEALHNHYTQKSLSLSPGK

SEQ ID NO: 11 - protein, 107 aa, Homo sapiens [sequence omitted]

SEQ ID NO: 12 - protein, 106 aa, Homo sapiens
GQPKAAPSVTLFPPSSEELQANKATLVCLISDFYPGAVTVAWKADSSPVKAGVETTTPSKQSNNKYAASSYLSLTPEQWKSHRSYSCQVTHEGSTVEKTVAPTECS

SEQ ID NO: 13 - protein, 118 aa, synthetic construct
EVQLVQSGAEVKKPGESLKISCKVSGYFFTTYWIGWVRQMPGKGLEYMGIIYPGDSDTRYSPSFQGQVTISADKSISTAYLQWSSLKASDTAMYYCARGGHWNAFDFWGQGTLVTVSS

SEQ ID NO: 14 - protein, 107 aa, synthetic construct
EIVLTQSPGTLSLSPGERATLSCRASQSVSSSYLAWYQQKPGQAPRLLIYGASRRATGIPDRFSGSGSGTDFTLTISRLEPEDFAVYYCQQFDASQTFGQGTKLEIS

SEQ ID NO: 15 - protein, 118 aa, synthetic construct
EVQLVQSGAEVKKPGESLKISCKVSGYFFTTYWIGWVRQMPGKGLEYMGIIYPGDSDTRYSPSFQGQVTISADKSISTAYLQWSSLKASDTAMYYCARGGNWNCFDYWGQGTLVTVSS

SEQ ID NO: 16 - protein, 107 aa, synthetic construct
EIVLTQSPGTLSLSPGERATLSCRASQSVSSSYLAWYQQKPGQAPRLLIYGASRRATGIPDRFSGSGSGTDFTLTISRLEPEDFAVYYCQRYGSSHTFGQGTKLEIS

SEQ ID NO: 17 - protein, 122 aa, synthetic construct
EVQLVESGGGLVQPGGSLRLSCAASEFTFSNYAMSWVRQAPGKGLEWVATISRGGDYTYYPDSVKGRFTISRDNSKNTLYLQMNSLRAEDTAVYYCARRVSMITGGWAMDYWGQGTLVTVSS

SEQ ID NO: 18 - protein, 112 aa, synthetic construct
DVVMTQSPLSLPVTLGQPASISCRSSQSIVDITGNTYLEWYQQRPGQSPRLLIYKVFNRFSGVPDRFSGSGSGTDFTLKISRVEAEDVGVYYCFQDSFVPYTFGQGTKLEIK

SEQ ID NO: 19 - protein, 118 aa, synthetic construct
EVQLVQSGAEVKKPGESLKISCKVSGYFFTTYWIGWVRQMPGKGLEYMGIIYPGDSDTRYSPSFQGQVTISADKSISTAYLQWSSLKASDTAMYYCARGGHWNAFDIWGQGTLVTVSS

SEQ ID NO: 20 - protein, 108 aa, synthetic construct
EIVLTQSPGTLSLSPGERATLSCRASQSVIGSYLAWYQQKPGQAPRLLIYSASKLASGIPDRFSGSGSGTDFTLTISRLEPEDFAVYYCQQHYSTPGTFGQGTKVEIK

SEQ ID NO: 21 - protein, 118 aa, synthetic construct
EVQLVQSGAEVKKPGESLKISCKVSGYFFTTYWIGWVRQMPGKGLEYMGIIYPGDSDTRYSPSFQGQVTISADKSISTAYLQWSSLKASDTAMYYCARGGHWNSFDTWGQGTLVTVSS

SEQ ID NO: 22 - protein, 117 aa, synthetic construct
QVTLKESGPVLVKPTETLTLTCTVSGFSLTTYAVHWIRQPPGKALEWLGVIWGAGSTDYNPSFMSRLTISKDTSKSQVVLTMTNMDPVDTATYYCAKNAAYYVMDYWGQGTTVTVSS

SEQ ID NO: 23 - protein, 108 aa, synthetic construct
EIVLTQSPGTLSLSPGERATLSCRASQSVIYSYLAWYQQKPGQAPRLLIYAASKLASGIPDRFSGSGSGTDFTLTISRLEPEDFAVYYCQQRASYPLTFGQGTKVEIK

SEQ ID NO: 24 - DNA, 19 bp, synthetic construct
  source 1..19: mol_type = other DNA
tgcatttgaactccttgcc

SEQ ID NO: 25 - DNA, 20 bp, synthetic construct
  source 1..20: mol_type = other DNA
ccatcaatcttccacttgac

SEQ ID NO: 26 - protein, 5 aa, synthetic construct
TYWIG

SEQ ID NO: 27 - protein, 17 aa, synthetic construct
IIYPGDSDTRYSPSFQG

SEQ ID NO: 28 - protein, 9 aa, synthetic construct
GGHWNAFDF

SEQ ID NO: 29 - protein, 9 aa, synthetic construct
GGHWNAFDI

SEQ ID NO: 30 - protein, 9 aa, synthetic construct
GGHWNSFDT

SEQ ID NO: 31 - protein, 5 aa, synthetic construct
TYAVH

SEQ ID NO: 32 - protein, 16 aa, synthetic construct
VIWGAGSTDYNPSFMS

SEQ ID NO: 33 - protein, 9 aa, synthetic construct
NAAYYVMDY

SEQ ID NO: 34 - protein, 12 aa, synthetic construct
RASQSVSSSYLA

SEQ ID NO: 35 - protein, 7 aa, synthetic construct
GASRRAT

SEQ ID NO: 36 - protein, 8 aa, synthetic construct
QQFDASQT

SEQ ID NO: 37 - protein, 12 aa, synthetic construct
RASQSVIGSYLA

SEQ ID NO: 38 - protein, 7 aa, synthetic construct
SASKLAS

SEQ ID NO: 39 - protein, 9 aa, synthetic construct
QQHYSTPGT

SEQ ID NO: 40 - protein, 12 aa, synthetic construct
RASQSVIYSYLA

SEQ ID NO: 41 - protein, 7 aa, synthetic construct
AASKLAS

SEQ ID NO: 42 - protein, 9 aa, synthetic construct
QQRASYPLT

SEQ ID NO: 43 - protein, 117 aa, synthetic construct
EVKLKESGPSLVQPSQSLSITCTVSGFSLTTYAVHWVRQSPGKGLEWLGVIWGAGSTDYNAAFMSRLSITKDNSKSQVFFKMNSLQADDTAIYFCAKNGAYYVMDYWGQGTSVTVSS

SEQ ID NO: 44 - protein, 106 aa, synthetic construct
EIVLTQSPAIMSASPGEKVTITCSASSSVSYMHWFQQRPGTSPKLWIYSTSNLASGVPARFSGSGSGTSYSLTISRMEAEDAATYYCQQRSSYPLTFGAGTKLEIK

SEQ ID NO: 45 - protein, 16 aa, synthetic construct
VIWGAGSTDYNAAFMS

SEQ ID NO: 46 - protein, 9 aa, synthetic construct
NGAYYVMDY

SEQ ID NO: 47 - protein, 10 aa, synthetic construct
SASSSVSYMH

SEQ ID NO: 48 - protein, 7 aa, synthetic construct
STSNLAS

SEQ ID NO: 49 - protein, 9 aa, synthetic construct
QQRSSYPLT

SEQ ID NO: 50 - protein, 115 aa, synthetic construct
EVQLLESGGGLVQPGGSLRLSCAASGFTFSSYAMSWVRQAPGKGLEWVSAISGSGGSTYYADSVKGRFTISRDNSKNTLYLQMNSLRAEDTAVYYCAKGSGFDYWGQGTLVTVSS

SEQ ID NO: 51 - protein, 108 aa, synthetic construct
EIVLTQSPGTLSLSPGERATLSCRASQSVSSSYLAWYQQKPGQAPRLLIYGASSRATGIPDRFSGSGSGTDFTLTISRLEPEDFAVYYCQQYGSSPLTFGQGTKVEIK